European Patent Specification EP 3 219 814 B1, published February 15, 2023. Title: PROBE FOR DETECTION OF POLYMORPHISM IN EGFR GENE, AMPLIFICATION PRIMER, AND USE THEREOF. Applicant: Arkray, Inc. The sequence listing filed with the application follows.

SEQUENCE LISTING (98 sequences)

SEQ ID NO: 1 - DNA, 410 bp, Homo sapiens
ctttccattctttggatcagtagtcactaacgttcgccagccataagtcctcgacgtggagaggctcagagcctggcatgaacatgaccctgaattcggatgcagagcttcttcccatgatgatctgtccctcacagcagggtcttctctgtttcagggcatgaactacttggaggaccgtcgcttggtgcaccgcgacctggcagccaggaacgtactggtgaaaacaccgcagcatgtcaagatcacagattttgggckggccaaacdgctgggtgcggaagagaaagaataccatgcagaaggaggcaaagtaaggaggtggctttaggtcagccagcattttcctgacaccagggaccaggctgccttcccactagctgtattgtttaacacatgcaggggaggat

SEQ ID NO: 2 - DNA, 287 bp, Homo sapiens
tcactgggcagcatgtggcaccatctcacaattgccagttaacgtcttccttctctctctgtcatagggactctggatcccagaaggtgagaaagttaaaattcccgtcgctatcaaggaattaagagaagcaacatctccgaaagccaacaaggaaatcctcgatgtgagtttctgctttgctgtgtgggggtccatggctctgaacctcaggcccaccttttctcatgtctggcagctgctctgctctagaccctgctcatctccacatcctaaatgttcacttt

SEQ ID NO: 3 - DNA, 272 bp, Homo sapiens
tcactgggcagcatgtggcaccatctcacaattgccagttaacgtcttccttctctctctgtcatagggactctggatcccagaaggtgagaaagttaaaattcccgtcgctatcaaggaattaagagaagcaacaaaggaaatcctcgatgtgagtttctgctttgctgtgtgggggtccatggctctgaacctcaggcccaccttttctcatgtctggcagctgctctgctctagaccctgctcatctccacatcctaaatgttcacttt

SEQ ID NO: 4 - DNA, 33 bp, Artificial
  probe
cccgtcgctatcaagtaattaagagaagcaaca

SEQ ID NO: 5 - DNA, 29 bp, Artificial
  probe
cccgtcgctatcaaggaattaagagaagc

SEQ ID NO: 6 - DNA, 16 bp, Artificial
  probe
agcaacaaaggaaatc

SEQ ID NO: 7 - DNA, 17 bp, Artificial
  probe
ttggcccgcccaaaatc

SEQ ID NO: 8 - DNA, 17 bp, Artificial
  probe
ttggccagcccaaaatc

SEQ ID NO: 9 - DNA, 15 bp, Artificial
  probe
cagtttggcccgccc

SEQ ID NO: 10 - DNA, 15 bp, Artificial
  probe
ctgtttggcccgccc

SEQ ID NO: 11 - DNA, 15 bp, Artificial
  probe
ccgtttggcccgccc

SEQ ID NO: 12 - DNA, 15 bp, Artificial
  probe
cagtttggccagccc

SEQ ID NO: 13 - DNA, 15 bp, Artificial
  probe
ctgtttggccagccc

SEQ ID NO: 14 - DNA, 15 bp, Artificial
  probe
ccgtttggccagccc

SEQ ID NO: 15 - DNA, 25 bp, Artificial
  primer
aggaacgtactggtgaaaacaccgc

SEQ ID NO: 16 - DNA, 28 bp, Artificial
  primer
ttactttgcctccttctgcatggtattc

SEQ ID NO: 17 - DNA, 27 bp, Artificial
  primer
gcctccttctgcatggtattctttctc

SEQ ID NO: 18 - DNA, 20 bp, Artificial
  primer
gatcccagaaggtgagaaag

SEQ ID NO: 19 - DNA, 20 bp, Artificial
  forward primer
tctctctgtcatagggactc

SEQ ID NO: 20 - DNA, 21 bp, Artificial
  reverse primer
gaaactcacatcgaggatttc

SEQ ID NO: 21 - DNA, 1020 bp, Homo sapiens
tggccactgttgcctgggcctctctgtcatggggaatccccagatgcacccaggaggggccctctcccactgcatctgtcacttcacagccctgcgtaaacgtccctgtgctaggtcttttgcaggcacagcttttcctccatgagtacgtattttgaaactcaagatcgcattcatgcgtcttcacctggaaggggtccatgtgcccctccttctggccaccatgcgaagccacactgacgtgcctctccctccctccaggaagcctacgtgatggccagcgtggacaacccccacgtgtgccgcctgctgggcatctgcctcacctccaccgtgcagctcatcaygcagctcatgcccttcggctgcctcctggactatgtccgggaacacaaagacaatattggctcccagtacctgctcaactggtgtgtgcagatcgcaaaggtaatcagggaagggagatacggggaggggagataaggagccaggatcctcacatgcggtctgcgctcctgggatagcaagagtttgccatggggatatgtgtgtgcgtgcatgcagcacacacacattcctttattttggattcaatcaagttgatcttcttgtgcacaaatcagtgcctgtcccatctgcatgtggaaactctcatcaatcagctacctttgaagaattttctctttattgagtgctcagtgtggtctgatgtctctgttcttatttctctggaattctttgtgaatactgtggtgatttgtagtggagaaggaatattgcttcccccattcaggacttgataacaaggtaagcaagccaggccaaggccaggaggacccaggtgatagtggtggagtggagcaggtgccttgcaggaggcccagtgaggaggtgcaaggagctgacagagggcgcagctgctgctgctatgtggctggggccttggctaagtgtccccctttccacaggctcgctccagagccagggcggggctgagagagcagagtggtcaggtagccc

SEQ ID NO: 22 - DNA, 22 bp, Artificial
  probe
tgagctgcrtgatgaggtgcac

SEQ ID NO: 23 - DNA, 22 bp, Artificial
  probe
tgagctgcatgatgaggtgcac

SEQ ID NO: 24 - DNA, 22 bp, Artificial
  probe
tgagctgcgtgatgaggtgcac

SEQ ID NO: 25 - DNA, 25 bp, Artificial
  foward primer
tccaggaagcctacgtgatggccag

SEQ ID NO: 26 - DNA, 32 bp, Artificial
  reverse primer
ccaatattgtctttgtgttcccggacatagtc

SEQ ID NO: 27 - DNA, 17 bp, Artificial
  probe
ccagcagtttggccagc

SEQ ID NO: 28 - DNA, 28 bp, Artificial
  probe
caaggaattaagagaagcaacatctccg

SEQ ID NO: 29 - DNA, 61 bp, Homo sapiens
cccgtcgctatcaaggaattaagagaagcaacatctccgaaagccaacaaggaaatcctcg

SEQ ID NO: 30 - DNA, 33 bp, Homo sapiens
cccgtcgctatcaaaacatctccgaaagccaac

SEQ ID NO: 31 - DNA, 45 bp, Homo sapiens
cccgtcgctatcaagacatctccgaaagccaaaaggaaatcctcg

SEQ ID NO: 32 - DNA, 50 bp, Homo sapiens
caagatcacagattttgggctggccaaactgctgggtgcggaagagaaag

SEQ ID NO: 33 - DNA, 50 bp, Homo sapiens
caagatcacagattttgggcgggccaaactgctgggtgcggaagagaaag

SEQ ID NO: 34 - DNA, 52 bp, Homo sapiens
cccgtcgctatcaaggaaccaacatctccgaaagccaacaaggaaatcctcg

SEQ ID NO: 35 - DNA, 46 bp, Homo sapiens
cccgtcgctatcaaggaatctccgaaagccaacaaggaaatcctcg

SEQ ID NO: 36 - DNA, 43 bp, Homo sapiens
cccgtcgctatcaaggaatcgaaagccaacaaggaaatcctcg

SEQ ID NO: 37 - DNA, 49 bp, Homo sapiens
cccgtcgctatcaaggaaccatctccgaaagccaacaaggaaatcctcg

SEQ ID NO: 38 - DNA, 43 bp, Homo sapiens
cccgtcgctatcaaggaaccgaaagccaacaaggaaatcctcg

SEQ ID NO: 39 - DNA, 43 bp, Homo sapiens
cccgtcgctatcaaggttccgaaagccaacaaggaaatcctcg

SEQ ID NO: 40 - DNA, 49 bp, Homo sapiens
cccgtcgctatcaaggaatcatctccgaaagccaacaaggaaatcctcg

SEQ ID NO: 41 - DNA, 43 bp, Homo sapiens; identical to SEQ ID NO: 36

SEQ ID NO: 42 - DNA, 43 bp, Homo sapiens
cccgtcgctatcaaggaacagaaagccaacaaggaaatcctcg

SEQ ID NO: 43 - DNA, 46 bp, Homo sapiens
cccgtcgctatcaaggtatctccgaaagccaacaaggaaatcctcg

SEQ ID NO: 44 - DNA, 43 bp, Homo sapiens; identical to SEQ ID NO: 39

SEQ ID NO: 45 - DNA, 44 bp, Homo sapiens
cccgtcgctatcaaaatctccgaaagccaacaaggaaatcctcg

SEQ ID NO: 46 - DNA, 46 bp, Homo sapiens
cccgtcgcaattaagatatctccgaaagccaacaaggaaatcctcg

SEQ ID NO: 47 - DNA, 46 bp, Homo sapiens
cccgtcgctatcaaggaacaaccgaaagccaacaaggaaatcctcg

SEQ ID NO: 48 - DNA, 46 bp, Homo sapiens
cccgtcgctatcaaggaattaagagaagcaacaaaggaaatcctcg

SEQ ID NO: 49 - DNA, 60 bp, Homo sapiens
ttccttgttggctttcggagatgttgcttctcttaattccttgatagcgacgggaatttt

SEQ ID NO: 50 - DNA, 60 bp, Homo sapiens
tcgaggatttccttgttggctttcggagatgttttgatagcgacgggaattttaactttc

SEQ ID NO: 51 - DNA, 60 bp, Homo sapiens
tcgaggatttccttgttggctttcggagatgtcttgatagcgacgggaattttaactttc

SEQ ID NO: 52 - DNA, 60 bp, Homo sapiens
gatttccttgttggctttcggagatgttggttccttgatagcgacgggaattttaacttt

SEQ ID NO: 53 - DNA, 60 bp, Homo sapiens
tcgaggatttccttgttggctttcggagattccttgatagcgacgggaattttaactttc

SEQ ID NO: 54 - DNA, 60 bp, Homo sapiens
atcgaggatttccttgttggctttcgattccttgatagcgacgggaattttaactttctc

SEQ ID NO: 55 - DNA, 60 bp, Homo sapiens
aggatttccttgttggctttcggagatggttccttgatagcgacgggaattttaactttc

SEQ ID NO: 56 - DNA, 60 bp, Homo sapiens
catcgaggatttccttgttggctttcggttccttgatagcgacgggaattttaactttct

SEQ ID NO: 57 - DNA, 60 bp, Homo sapiens
catcgaggatttccttgttggctttcggaaccttgatagcgacgggaattttaactttct

SEQ ID NO: 58 - DNA, 60 bp, Homo sapiens
ggatttccttgttggctttcggagatgattccttgatagcgacgggaattttaactttct

SEQ ID NO: 59 - DNA, 60 bp, Homo sapiens
catcgaggatttccttgttggctttcgattccttgatagcgacgggaattttaactttct

SEQ ID NO: 60 - DNA, 60 bp, Homo sapiens
catcgaggatttccttgttggctttctgttccttgatagcgacgggaattttaactttct

SEQ ID NO: 61 - DNA, 60 bp, Homo sapiens
tcgaggatttccttgttggctttcggagataccttgatagcgacgggaattttaactttc

SEQ ID NO: 62 - DNA, 60 bp, Homo sapiens
acatcgaggatttccttgttggctttcggaaccttgatagcgacgggaattttaactttc

SEQ ID NO: 63 - DNA, 60 bp, Homo sapiens
acatcgaggatttccttgttggctttcggaattttgatagcgacgggaattttaactttc

SEQ ID NO: 64 - DNA, 60 bp, Homo sapiens
tcgaggatttccttgttggctttcggagatatcttaattgcgacgggaattttaactttc

SEQ ID NO: 65 - DNA, 60 bp, Homo sapiens
tcgaggatttccttgttggctttcggttgttccttgatagcgacgggaattttaactttc

SEQ ID NO: 66 - DNA, 60 bp, Homo sapiens
cgaggatttcctttgttgcttctcttaattccttgatagcgacgggaattttaactttct

SEQ ID NO: 67 - DNA, 90 bp, Artificial
  oligonucleotide
actggtgaaaacaccgcagcatgtcaagatcacagattttgggctggccaaactgctgggtgcggaagagaaagaataccatgcagaagg

SEQ ID NO: 68 - DNA, 90 bp, Artificial
  oligonucleotide
actggtgaaaacaccgcagcatgtcaagatcacagattttgggcgggccaaactgctgggtgcggaagagaaagaataccatgcagaagg

SEQ ID NO: 69 - DNA, 90 bp, Artificial
  oligonucleotide
ccttctgcatggtattctttctcttccgcacccagcagtttggccagcccaaaatctgtgatcttgacatgctgcggtgttttcaccagt

SEQ ID NO: 70 - DNA, 90 bp, Artificial
  oligonucleotide
ccttctgcatggtattctttctcttccgcacccagcagtttggcccgcccaaaatctgtgatcttgacatgctgcggtgttttcaccagt

SEQ ID NO: 71 - DNA, 31 bp, Artificial
  probe
ccgcccaaaatctgtgatcttgacatgctgc

SEQ ID NO: 72 - DNA, 30 bp, Artificial
  probe
gcccgcccaaaatctgtgatcttgacatgc

SEQ ID NO: 73 - DNA, 26 bp, Artificial
  probe
gcccgcccaaaatctgtgatcttgac

SEQ ID NO: 74 - DNA, 23 bp, Artificial
  probe
tggcccgcccaaaatctgtgatc

SEQ ID NO: 75 - DNA, 16 bp, Artificial
  probe
agcagtttggcccgcc

SEQ ID NO: 76 - DNA, 19 bp, Artificial
  probe
acccagcagtttggcccgc

SEQ ID NO: 77 - DNA, 18 bp, Artificial
  probe
cccgcccaaaatctgtga

SEQ ID NO: 78 - DNA, 18 bp, Artificial
  probe
ccgcccaaaatctgtgat

SEQ ID NO: 79 - DNA, 22 bp, Artificial
  perobe
cagtttggcccgcccaaaatct

SEQ ID NO: 80 - DNA, 22 bp, Artificial
  probe
cagcagtttggcccgcccaaaa

SEQ ID NO: 81 - DNA, 23 bp, Artificial
  probe
ccagcagtttggcccgcccaaaa

SEQ ID NO: 82 - DNA, 24 bp, Artificial
  probe
cccagcagtttggcccgcccaaaa

SEQ ID NO: 83 - DNA, 24 bp, Artificial
  probe
cacccagcagtttggcccgcccaa

SEQ ID NO: 84 - DNA, 24 bp, Artificial
  probe
cgcacccagcagtttggcccgccc

SEQ ID NO: 85 - DNA, 24 bp, Artificial
  probe
ccgcacccagcagtttggcccgcc

SEQ ID NO: 86 - DNA, 27 bp, Artificial
  probe
cttccgcacccagcagtttggcccgcc

SEQ ID NO: 87 - DNA, 31 bp, Artificial
  probe
ctttctcttccgcacccagcagtttggcccg

SEQ ID NO: 88 - DNA, 18 bp, Artificial
  probe
cagcagtttggcccgccc

SEQ ID NO: 89 - DNA, 29 bp, Artificial
  probe
catgtcaagatcacagattttgggcgggc

SEQ ID NO: 90 - DNA, 24 bp, Artificial
  probe
caagatcacagattttgggcgggc

SEQ ID NO: 91 - DNA, 22 bp, Artificial
  probe
cacagattttgggcgggccaaa

SEQ ID NO: 92 - DNA, 20 bp, Artificial
  probe
cagattttgggcgggccaaa

SEQ ID NO: 93 - DNA, 20 bp, Artificial
  probe
cgggccaaactgctgggtgc

SEQ ID NO: 94 - DNA, 20 bp, Artificial
  probe
atcacagattttgggcgggc

SEQ ID NO: 95 - DNA, 21 bp, Artificial
  probe
atcacagattttgggcgggcc

SEQ ID NO: 96 - DNA, 18 bp, Artificial
  probe
attttgggcgggccaaac

SEQ ID NO: 97 - DNA, 21 bp, Artificial
  probe
attttgggcgggccaaactgc

SEQ ID NO: 98 - DNA, 22 bp, Artificial
  probe
ggcgggccaaactgctgggtgc